European Patent Application EP 4 506 341 A1, published February 12, 2025. Title: TISSUE REGENERATION APPROACHES. Applicant: ZeCardio Therapeutics SL. The sequence listing filed with the application follows.

SEQUENCE LISTING (15 sequences)

SEQ ID NO: 1 - DNA, 22 bp, synthetic construct
  source 1..22: mol_type = other DNA; note = Tob1a forward primer sequence
atgcagcttgaaatccaagtag

SEQ ID NO: 2 - DNA, 18 bp, synthetic construct
  source 1..18: mol_type = other DNA; note = Tob1a reverse primer sequence
gttggccatcactggctg

SEQ ID NO: 3 - DNA, 20 bp, synthetic construct
  source 1..20: mol_type = other DNA; note = Tob1 sgRNA1 sequence
aaaaatgttgacacgtctcc

SEQ ID NO: 4 - DNA, 20 bp, synthetic construct
  source 1..20: mol_type = other DNA; note = Tob1 sgRNA2 sequence
gttaaaggctgagtggaccg

SEQ ID NO: 5 - RNA, 16 nt, synthetic construct
  source 1..16: mol_type = other RNA; note = Negative control sequence
gcactaccagagctaa

SEQ ID NO: 6 - DNA, 23 bp, synthetic construct
  source 1..23: mol_type = other DNA; note = Tob1 forward primer sequence
tttgtttctctgccacaaactga

SEQ ID NO: 7 - DNA, 20 bp, synthetic construct
  source 1..20: mol_type = other DNA; note = Tob1 reverse primer sequence
ctgaggttaagggggctgtc

SEQ ID NO: 8 - DNA, 21 bp, synthetic construct
  source 1..21: mol_type = other DNA; note = Cdk1 forward primer sequence
gatctgtaaggaccagctcac

SEQ ID NO: 9 - DNA, 22 bp, synthetic construct
  source 1..22: mol_type = other DNA; note = Cdk1 reverse primer sequence
ccataagtcccttctccgattt

SEQ ID NO: 10 - DNA, 20 bp, synthetic construct
  source 1..20: mol_type = other DNA; note = Ccnb1 forward primer sequence
gccagaggttagggtgtctt

SEQ ID NO: 11 - DNA, 20 bp, synthetic construct
  source 1..20: mol_type = other DNA; note = Ccnb1 reverse primer sequence
agttctcgatctcagcaggg

SEQ ID NO: 12 - DNA, 21 bp, synthetic construct
  source 1..21: mol_type = other DNA; note = Gadph forward primer sequence
actcccattcttccacctttg

SEQ ID NO: 13 - DNA, 21 bp, synthetic construct
  source 1..21: mol_type = other DNA; note = Gapdh reverse primer sequence
ccctgttgctgtagccatatt

SEQ ID NO: 14 - DNA, 21 bp, synthetic construct
  source 1..21: mol_type = other DNA; note = Tob1 forward primer sequence
gaaccacagcagccatttgtg

SEQ ID NO: 15 - DNA, 20 bp, synthetic construct
  source 1..20: mol_type = other DNA; note = Tob1 reverse primer sequence
aaccacatggttcaccctcg